European Patent Specification EP 3 801 029 B1, published July 10, 2024. Title: ANTIBACTERIAL COMPOSITIONS, METHODS OF MAKING AND USE THEREOF. Applicant: Morehouse School of Medicine. Application US 16/226,242. The sequence listing filed with the application follows.

SEQUENCE LISTING (11 sequences)

SEQ ID NO: 1 - protein, 5 aa, Human immunodeficiency virus
VGFPV

SEQ ID NO: 2 - protein, 5 aa, Simian immunodeficiency virus
VGVSV

SEQ ID NO: 3 - protein, 12 aa, Human immunodeficiency virus
VGFPVAAVGFPV

SEQ ID NO: 4 - protein, 12 aa, ARTIFICIAL SEQUENCE
  Synthetic
VGVSVAAVGVSV

SEQ ID NO: 5 - protein, 20 aa, ARTIFICIAL SEQUENCE
  Synthetic
VGFPVAAVGFPVDYKDDDDK

SEQ ID NO: 6 - protein, 8 aa, ARTIFICIAL SEQUENCE
  Synthetic
DYKDDDDK

SEQ ID NO: 7 - protein, 20 aa, ARTIFICIAL SEQUENCE
  Synthetic
AGFPVAAAGFPVDYKDDDDK

SEQ ID NO: 8 - protein, 13 aa, Human immunodeficiency virus
GRKKRRQRRRPPQ

SEQ ID NO: 9 - protein, 25 aa, ARTIFICIAL SEQUENCE
  Synthetic
VGFPVAAVGFPVGRKKRRQRRRPPQ

SEQ ID NO: 10 - protein, 12 aa, ARTIFICIAL SEQUENCE
  Synthetic
AGFPVAAAGFPV

SEQ ID NO: 11 - protein, 25 aa, ARTIFICIAL SEQUENCE
  Synthetic
AGFPVAAAGFPVGRKKRRQRRRPPQ